European Patent Application EP 4 703 373 A1, published March 4, 2026. Title: POLYPEPTIDES AND RELATED SUBSTANCES AGAINST HAIR LOSS AND DERMATITIS, AND USES THEREOF. Applicant: SHENZHEN INSTITUTES OF ADVANCED TECHNOLOGY. Application WO PCT/CN2023/090364, filed April 24, 2023. The sequence listing filed with the application follows.

SEQUENCE LISTING (9 sequences)

SEQ ID NO: 1 - protein, 19 aa, Homo
YLYQWLGAPVPYPDPLEPR

SEQ ID NO: 2 - protein, 15 aa, Mus
YLGASVPSPDPLEPT

SEQ ID NO: 3 - protein, 18 aa, Ovis/Lutra/Lontra/Meles
LDPGLGAPAPYPDPLEPR

SEQ ID NO: 4 - protein, 20 aa, Podarcis/Zootoca
NYNRFYNARAAPTPDPLEPL

SEQ ID NO: 5 - protein, 19 aa, Lithobates
SNLRNAVFGTPVRDPLESK

SEQ ID NO: 6 - protein, 17 aa, Megalobram
AGAVTAADLSLTQLESL

SEQ ID NO: 7 - protein, 18 aa, Gallus
YAQDSGVAGAPPNPLEAQ

SEQ ID NO: 8 - protein, 18 aa, Aix/Anser
SDFYERYFMHYKTPMEQM

SEQ ID NO: 9 - protein, 15 aa, unidentified
DHTLVFSNERWPGVS